European Patent Specification EP 4 188 410 B1, published November 5, 2025. Title: CHIMERIC PROTEINS AND METHODS OF USE FOR TREATMENT OF CENTRAL NERVOUS SYSTEM DISORDERS. Applicant: Silver Creek Pharmaceuticals, Inc. Application PCT/US2021/044019. The sequence listing filed with the application follows.

SEQUENCE LISTING (25 sequences)

SEQ ID NO: 1 - protein, 70 aa, Homo sapiens
GPETLCGAELVDALQFVCGDRGFYFNKPTGYGSSSRRAPQTGIVDECCFRSCDLRRLEMYCAPLKPAKSA

SEQ ID NO: 2 - protein, 70 aa, Artificial Sequence
  synthetic construct
GPRTLCGAELVDALQFVCGDRGFYFNKPTGAGSSSRRAPQTGIVDECCFRSCDLRRLEMYCAPLKPAKSA

SEQ ID NO: 3 - protein, 83 aa, Artificial Sequence
  synthetic construct
MFPAMPLSSLFVNGPETLCGAELVDALQFVCGDRGFYFNKPTGYGSSSRRAPQTGIVDECCFRSCDLRRLEMYCAPLKPAKSA

SEQ ID NO: 4 - protein, 70 aa, Artificial Sequence
  synthetic construct
GPRTLCGAELVDALQFVCGDRGFYFNKPTGYGSSSRRAPQTGIVDECCFRSCDLRRLEMYCAPLKPAKSA

SEQ ID NO: 5 - protein, 67 aa, Artificial Sequence
  synthetic construct
TLCGAELVDALQFVCGDRGFYFNKPTGYGSSSRRAPQTGIVDECCFRSCDLRRLEMYCAPLKPAKSA

SEQ ID NO: 6 - protein, 83 aa, Artificial Sequence
  synthetic construct
MFPAMPLSSLFVNGPRTLCGAELVDALQFVCGDRGFYFNKPTGYGSSSRRAPQTGIVDECCFRSCDLRRLEMYCAPLKPAKSA

SEQ ID NO: 7 - protein, 69 aa, Artificial Sequence
  synthetic construct
GPETLCGAELVDALQFVCGDRGFYFNKPTGYGSSSRAPQTGIVDECCFRSCDLRRLEMYCAPLKPAKSA

SEQ ID NO: 8 - protein, 67 aa, Artificial Sequence
  synthetic construct
GPETLCGAELVDALQFVCGDRGFYFNKPTGYGSSSRRAPQTGIVDECCFRSCDLRRLEMYCAPLKPA

SEQ ID NO: 9 - protein, 319 aa, Homo sapiens
AQVLRGTVTDFPGFDERADAETLRKAMKGLGTDEESILTLLTSRSNAQRQEISAAFKTLFGRDLLDDLKSELTGKFEKLIVALMKPSRLYDAYELKHALKGAGTNEKVLTEIIASRTPEELRAIKQVYEEEYGSSLEDDVVGDTSGYYQRMLVVLLQANRDPDAGIDEAQVEQDAQALFQAGELKWGTDEEKFITIFGTRSVSHLRKVFDKYMTISGFQIEETIDRETSGNLEQLLLAVVKSIRSIPAYLAETLYYAMKGAGTDDHTLIRVMVSRSEIDLFNIRKEFRKNFATSLYSMIKGDTSGDYKKALLLLCGEDD

SEQ ID NO: 10 - protein, 319 aa, Artificial Sequence
  synthetic construct
AQVLRGTVTDFPGFDERADAETLRKAMKGLGTDEESILTLLTSRSNAQRQEISAAFKTLFGADLLDDLASELTGKFEKLIVALMKPSRLYDAYELKHALAGAGTNEKVLTEIIASRTPEELRAIKQVYEEEYGSSLAGDVVGDTSGYYQRMLVVLLQAARDPDAGIDEAQVEQDAQALFQAGELKWGTDEEKFITIFGTRSVSHLRKVFDKYMTISGFQIEETIDRETSGNLEQLLLAVVKSIRSIPAYLAETLYYAMKGAGTDDHTLIRVMVSRSEIDLFNIRKEFRKNFATSLYSMIKGDTSGDYKKALLLLAGEDD

SEQ ID NO: 11 - protein, 319 aa, Artificial Sequence
  synthetic construct
AQVLRGTVTDFPGFDERADAETLRKAMKGLGTDEESILTLLTSRSNAQRQEISAAFKTLFGADLLDDLASELTGKFEKLIVALMKPSRLYDAYELKHALAGAGTNEKVLTEIIASRTPEELRAIKQVYEEEYGSSLAGDVVGDTSGYYQRMLVVLLQAARDPDAGIDEAQVEQDAQALFQAGELKWGTDEEKFITIFGTRSVSHLRKVFDKYMTISGFQIEETIDRETSGNLEQLLLAVVKSIRSIPAYLAETLYYAMKGAGTDDHTLIRVMVSRSEIDLFNIRKEFRKNFATSLYSMIKGDTSGDYKKALLLLCGEDD

SEQ ID NO: 12 - protein, 585 aa, Homo sapiens [sequence omitted]

SEQ ID NO: 13 - protein, 585 aa, Artificial Sequence
  synthetic construct
DAHKSEVAHRFKDLGEENFKALVLIAFAQYLQQSPFEDHVKLVNEVTEFAKTCVADESAENCDKSLHTLFGDKLCTVATLRETYGEMADCCAKQEPERNECFLQHKDDNPNLPRLVRPEVDVMCTAFHDNEETFLKKYLYEIARRHPYFYAPELLFFAKRYKAAFTECCQAADKAACLLPKLDELRDEGKASSAKQRLKCASLQKFGERAFKAWAVARLSQRFPKAEFAEVSKLVTDLTKVHTECCHGDLLECADDRADLAKYICENQDSISSKLKECCEKPLLEKSHCIAEVENDEMPADLPSLAADFVESKDVCKNYAEAKDVFLGMFLYEYARRHPDYSVVLLLRLAKTYETTLEKCCAAADPHECYAKVFDEFKPLVEEPQNLIKQNCELFEQLGEYKFQNALLVRYTKKVPQVSTPTLVEVSRNLGKVGSKCCKHPEAKRMPCAEDYLSVVLNQLCVLHEKTPVSDRVTKCCTESLVNRRPCFSALEVDETYVPKEFQAETFTFHADICTLSEKERQIKKQTALVELVKHKPKATKEQLKAVMDDFAAFVEKCCKADDKETCFAEEGKKLVAASQAALGL

SEQ ID NO: 14 - protein, 585 aa, Artificial Sequence
  synthetic construct
DAHKSEVAHRFKDLGEENFKALVLIAFAQYLQQSPFEDHVKLVNEVTEFAKTCVADESAENCDKSLHTLFGDKLCTVATLRETYGEMADCCAKQEPERNECFLQHKDDNPNLPRLVRPEVDVMCTAFHDNEETFLKKYLYEIARRHPYFYAPELLFFAKRYKAAFTECCQAADKAACLLPKLDELRDEGKASSAKQRLKCASLQKFGERAFKAWAVARLSQRFPKAEFAEVSKLVTDLTKVHTECCHGDLLECADDRADLAKYICENQDSISSKLKECCEKPLLEKSHCIAEVENDEMPADLPSLAADFVESKDVCKNYAEAKDVFLGMFLYEYARRHPDYSVVLLLRLAKTYETTLEKCCAAADPHECYAKVFDEFKPLVEEPQNLIKQNCELFEQLGEYKFQNALLVRYTKKVPQVSTPTLVEVSRNLGKVGSKCCKHPEAKRMPCAEDYLSVVLNQLCVLHEKTPVSDRVTKCCTESLVNRRPCFSALEVDETYVPKEFQAGTFTFHADICTLSEKERQIKKQTALVELVKHKPKATKEQLKAAMDDFAAFVEKCCKADDKETCFAEEGKKLVAASQAALGL

SEQ ID NO: 15 - protein, 585 aa, Artificial Sequence; identical to SEQ ID NO: 13
  synthetic construct

SEQ ID NO: 16 - protein, 20 aa, Artificial Sequence
  synthetic construct
GGGGSGGGGSGGGGSGGGGS

SEQ ID NO: 17 - protein, 698 aa, Homo sapiens
MRLAVGALLVCAVLGLCLAVPDKTVRWCAVSEHEATKCQSFRDHMKSVIPSDGPSVACVKKASYLDCIRAIAANEADAVTLDAGLVYDAYLAPNNLKPVVAEFYGSKEDPQTFYYAVAVVKKDSGFQMNQLRGKKSCHTGLGRSAGWNIPIGLLYCDLPEPRKPLEKAVANFFSGSCAPCADGTDFPQLCQLCPGCGCSTLNQYFGYSGAFKCLKDGAGDVAFVKHSTIFENLANKADRDQYELLCLDNTRKPVDEYKDCHLAQVPSHTVVARSMGGKEDLIWELLNQAQEHFGKDKSKEFQLFSSPHGKDLLFKDSAHGFLKVPPRMDAKMYLGYEYVTAIRNLREGTCPEAPTDECKPVKWCALSHHERLKCDEWSVNSVGKIECVSAETTEDCIAKIMNGEADAMSLDGGFVYIAGKCGLVPVLAENYNKSDNCEDTPEAGYFAIAVVKKSASDLTWDNLKGKKSCHTAVGRTAGWNIPMGLLYNKINHCRFDEFFSEGCAPGSKKDSSLCKLCMGSGLNLCEPNNKEGYYGYTGAFRCLVEKGDVAFVKHQTVPQNTGGKNPDPWAKNLNEKDYELLCLDGTRKPVEEYANCHLARAPNHAVVTRKDKEACVHKILRQQQHLFGSNVTDCSGNFCLFRSETKDLLFRDDTVCLAKLHDRNTYEKYLGEEYVKAVGNLRKCSTSSLLEACTFRRP

SEQ ID NO: 18 - protein, 609 aa, Homo sapiens
MKWVESIFLIFLLNFTESRTLHRNEYGIASILDSYQCTAEISLADLATIFFAQFVQEATYKEVSKMVKDALTAIEKPTGDEQSSGCLENQLPAFLEELCHEKEILEKYGHSDCCSQSEEGRHNCFLAHKKPTPASIPLFQVPEPVTSCEAYEEDRETFMNKFIYEIARRHPFLYAPTILLWAARYDKIIPSCCKAENAVECFQTKAATVTKELRESSLLNQHACAVMKNFGTRTFQAITVTKLSQKFTKVNFTEIQKLVLDVAHVHEHCCRGDVLDCLQDGEKIMSYICSQQDTLSNKITECCKLTTLERGQCIIHAENDEKPEGLSPNLNRFLGDRDFNQFSSGEKNIFLASFVHEYSRRHPQLAVSVILRVAKGYQELLEKCFQTENPLECQDKGEEELQKYIQESQALAKRSCGLFQKLGEYYLQNAFLVAYTKKAPQLTSSELMAITRKMAATAATCCQLSEDKLLACGEGAADIIIGHLCIRHEMTPVNPGVGQCCTSSYANRRPCFSSLVVDETYVPPAFSDDKFIFHKDLCQAQGVALQTMKQEFLINLVKQKPQITEEQLEAVIADFSGLLEKCCQGQEQEVCFAEEGQKLISKTRAALGV

SEQ ID NO: 19 - protein, 474 aa, Homo sapiens
MKRVLVLLLAVAFGHALERGRDYEKNKVCKEFSHLGKEDFTSLSLVLYSRKFPSGTFEQVSQLVKEVVSLTEACCAEGADPDCYDTRTSALSAKSCESNSPFPVHPGTAECCTKEGLERKLCMAALKHQPQEFPTYVEPTNDEICEAFRKDPKEYANQFMWEYSTNYGQAPLSLLVSYTKSYLSMVGSCCTSASPTVCFLKERLQLKHLSLLTTLSNRVCSQYAAYGEKKSRLSNLIKLAQKVPTADLEDVLPLAEDITNILSKCCESASEDCMAKELPEHTVKLCDNLSTKNSKFEDCCQEKTAMDVFVCTYFMPAAQLPELPDVELPTNKDVCDPGNTKVMDKYTFELSRRTHLPEVFLSKVLEPTLKSLGECCDVEDSTTCFNAKGPLLKKELSSFIDKGQELCADYSENTFTEYKKKLAERLKAKLPDATPTELAKLVNKHSDFASNCCSINSPPLYCDSEIDAELKNIL

SEQ ID NO: 20 - protein, 147 aa, Homo sapiens
MASHRLLLLCLAGLVFVSEAGPTGTGESKCPLMVKVLDAVRGSPAINVAVHVFRKAADDTWEPFASGKTSESGELHGLTTEEEFVEGIYKVEIDTKSYWKALGISPFHEHAEVVFTANDSGPRRYTIAALLSPYSYSTTAVVTNPKE

SEQ ID NO: 21 - protein, 20 aa, Artificial Sequence
  synthetic construct
ASPAAPAPASPAAPAPSAPA

SEQ ID NO: 22 - protein, 107 aa, Artificial Sequence
  synthetic construct
DIQMTQSPSSLSASVGDRVTITCRASQWIGSQLSWYQQKPGKAPKLLIMWRSSLQSGVPSRFSGSGSGTDFTLTISSLQPEDFATYYCAQGAALPRTFGQGTKVEIK

SEQ ID NO: 23 - protein, 7 aa, Artificial Sequence
  synthetic construct
GSGGGSG

SEQ ID NO: 24 - protein, 988 aa, Artificial Sequence
  synthetic construct
GPRTLCGAELVDALQFVCGDRGFYFNKPTGAGSSSRRAPQTGIVDECCFRSCDLRRLEMYCAPLKPAKSAGSGGGSGDAHKSEVAHRFKDLGEENFKALVLIAFAQYLQQSPFEDHVKLVNEVTEFAKTCVADESAENCDKSLHTLFGDKLCTVATLRETYGEMADCCAKQEPERNECFLQHKDDNPNLPRLVRPEVDVMCTAFHDNEETFLKKYLYEIARRHPYFYAPELLFFAKRYKAAFTECCQAADKAACLLPKLDELRDEGKASSAKQRLKCASLQKFGERAFKAWAVARLSQRFPKAEFAEVSKLVTDLTKVHTECCHGDLLECADDRADLAKYICENQDSISSKLKECCEKPLLEKSHCIAEVENDEMPADLPSLAADFVESKDVCKNYAEAKDVFLGMFLYEYARRHPDYSVVLLLRLAKTYETTLEKCCAAADPHECYAKVFDEFKPLVEEPQNLIKQNCELFEQLGEYKFQNALLVRYTKKVPQVSTPTLVEVSRNLGKVGSKCCKHPEAKRMPCAEDYLSVVLNQLCVLHEKTPVSDRVTKCCTESLVNRRPCFSALEVDETYVPKEFQAETFTFHADICTLSEKERQIKKQTALVELVKHKPKATKEQLKAVMDDFAAFVEKCCKADDKETCFAEEGKKLVAASQAALGLGSGGGSGAQVLRGTVTDFPGFDERADAETLRKAMKGLGTDEESILTLLTSRSNAQRQEISAAFKTLFGADLLDDLASELTGKFEKLIVALMKPSRLYDAYELKHALAGAGTNEKVLTEIIASRTPEELRAIKQVYEEEYGSSLAGDVVGDTSGYYQRMLVVLLQAARDPDAGIDEAQVEQDAQALFQAGELKWGTDEEKFITIFGTRSVSHLRKVFDKYMTISGFQIEETIDRETSGNLEQLLLAVVKSIRSIPAYLAETLYYAMKGAGTDDHTLIRVMVSRSEIDLFNIRKEFRKNFATSLYSMIKGDTSGDYKKALLLLAGEDD

SEQ ID NO: 25 - protein, 988 aa, Artificial Sequence
  Synthetic construct
GPRTLCGAELVDALQFVCGDRGFYFNKPTGAGSSSRRAPQTGIVDECCFRSCDLRRLEMYCAPLKPAKSAGSGGGSGDAHKSEVAHRFKDLGEENFKALVLIAFAQYLQQSPFEDHVKLVNEVTEFAKTCVADESAENCDKSLHTLFGDKLCTVATLRETYGEMADCCAKQEPERNECFLQHKDDNPNLPRLVRPEVDVMCTAFHDNEETFLKKYLYEIARRHPYFYAPELLFFAKRYKAAFTECCQAADKAACLLPKLDELRDEGKASSAKQRLKCASLQKFGERAFKAWAVARLSQRFPKAEFAEVSKLVTDLTKVHTECCHGDLLECADDRADLAKYICENQDSISSKLKECCEKPLLEKSHCIAEVENDEMPADLPSLAADFVESKDVCKNYAEAKDVFLGMFLYEYARRHPDYSVVLLLRLAKTYETTLEKCCAAADPHECYAKVFDEFKPLVEEPQNLIKQNCELFEQLGEYKFQNALLVRYTKKVPQVSTPTLVEVSRNLGKVGSKCCKHPEAKRMPCAEDYLSVVLNQLCVLHEKTPVSDRVTKCCTESLVNRRPCFSALEVDETYVPKEFQAETFTFHADICTLSEKERQIKKQTALVELVKHKPKATKEQLKAVMDDFAAFVEKCCKADDKETCFAEEGKKLVAASQAALGLGSGGGSGAQVLRGTVTDFPGFDERADAETLRKAMKGLGTDEESILTLLTSRSNAQRQEISAAFKTLFGADLLDDLASELTGKFEKLIVALMKPSRLYDAYELKHALAGAGTNEKVLTEIIASRTPEELRAIKQVYEEEYGSSLAGDVVGDTSGYYQRMLVVLLQAARDPDAGIDEAQVEQDAQALFQAGELKWGTDEEKFITIFGTRSVSHLRKVFDKYMTISGFQIEETIDRETSGNLEQLLLAVVKSIRSIPAYLAETLYYAMKGAGTDDHTLIRVMVSRSEIDLFNIRKEFRKNFATSLYSMIKGDTSGDYKKALLLLSGEDD